European Patent Application EP 4 174 177 A1, published May 3, 2023. Title: Coronavirus specific siRNA and a composition for preventing and treating coronavirus infection-19 comprising the same. Applicant: Agency of Defense Development LOGONE Bio-Convergence Research Foundation. The sequence listing filed with the application follows.

SEQUENCE LISTING (122 sequences)

SEQ ID NO: 1 - RNA, 19 nt, Artificial Sequence
  Severe acute respiratory syndrome coronavirus 2
cuuguagaucuguucucua

SEQ ID NO: 2 - RNA, 19 nt, Artificial Sequence
  Severe acute respiratory syndrome coronavirus 2
cucuaaacgaacuuuaaaa

SEQ ID NO: 3 - RNA, 19 nt, Artificial Sequence
  Severe acute respiratory syndrome coronavirus 2
cuugaauacaccaaaagau

SEQ ID NO: 4 - RNA, 19 nt, Artificial Sequence
  Severe acute respiratory syndrome coronavirus 2
cugguaaaggccaacaaca

SEQ ID NO: 5 - RNA, 19 nt, Artificial Sequence
  Severe acute respiratory syndrome coronavirus 2
caaacugucacuaagaaau

SEQ ID NO: 6 - RNA, 19 nt, Artificial Sequence
  Severe acute respiratory syndrome coronavirus 2
caaagauccaaauuucaaa

SEQ ID NO: 7 - RNA, 19 nt, Artificial Sequence
  Severe acute respiratory syndrome coronavirus 2
cuaaaaaggacaaaaagaa

SEQ ID NO: 8 - RNA, 19 nt, Artificial Sequence
  Severe acute respiratory syndrome coronavirus 2
cauaaucaggauguaaacu

SEQ ID NO: 9 - RNA, 19 nt, Artificial Sequence
  Severe acute respiratory syndrome coronavirus 2
caauguugcuuuucaaacu

SEQ ID NO: 10 - RNA, 19 nt, Artificial Sequence
  Severe acute respiratory syndrome coronavirus 2
cuuuaaggaaggaaguucu

SEQ ID NO: 11 - RNA, 19 nt, Artificial Sequence
  Severe acute respiratory syndrome coronavirus 2
gaguuaugaggaucaagau

SEQ ID NO: 12 - RNA, 19 nt, Artificial Sequence
  Severe acute respiratory syndrome coronavirus 2
ccuacuauaacucaaauga

SEQ ID NO: 13 - RNA, 19 nt, Artificial Sequence
  Severe acute respiratory syndrome coronavirus 2
cauuagugcaaagaauaga

SEQ ID NO: 14 - RNA, 19 nt, Artificial Sequence
  Severe acute respiratory syndrome coronavirus 2
ggaguaugcugaugucuuu

SEQ ID NO: 15 - RNA, 19 nt, Artificial Sequence
  Severe acute respiratory syndrome coronavirus 2
cuaagguuggugguaauua

SEQ ID NO: 16 - RNA, 19 nt, Artificial Sequence
  Severe acute respiratory syndrome coronavirus 2
ccuuuugagagagauauuu

SEQ ID NO: 17 - RNA, 19 nt, Artificial Sequence
  Severe acute respiratory syndrome coronavirus 2
gauuuuggugguuuuaauu

SEQ ID NO: 18 - RNA, 19 nt, Artificial Sequence
  Severe acute respiratory syndrome coronavirus 2
cuuuaaacacgcuuguuaa

SEQ ID NO: 19 - RNA, 19 nt, Artificial Sequence
  Severe acute respiratory syndrome coronavirus 2
guaaacauucaaaaagaaa

SEQ ID NO: 20 - RNA, 19 nt, Artificial Sequence
  Severe acute respiratory syndrome coronavirus 2
caagaauuuaaaugaaucu

SEQ ID NO: 21 - RNA, 19 nt, Artificial Sequence
  Severe acute respiratory syndrome coronavirus 2
gaaaguaugagcaguauau

SEQ ID NO: 22 - RNA, 19 nt, Artificial Sequence
  Severe acute respiratory syndrome coronavirus 2
cuuguggcuuaguagaagu

SEQ ID NO: 23 - RNA, 19 nt, Artificial Sequence
  Severe acute respiratory syndrome coronavirus 2
cagcccuauguguucauca

SEQ ID NO: 24 - RNA, 19 nt, Artificial Sequence
  Severe acute respiratory syndrome coronavirus 2
cuacccucuugagugcauu

SEQ ID NO: 25 - RNA, 19 nt, Artificial Sequence
  Severe acute respiratory syndrome coronavirus 2
cauuagaacaaccuacuag

SEQ ID NO: 26 - RNA, 19 nt, Artificial Sequence
  Severe acute respiratory syndrome coronavirus 2
ggaccugagcauagucuug

SEQ ID NO: 27 - RNA, 19 nt, Artificial Sequence
  Severe acute respiratory syndrome coronavirus 2
gcccuugcaccuaauauga

SEQ ID NO: 28 - RNA, 19 nt, Artificial Sequence
  Severe acute respiratory syndrome coronavirus 2
cauuccaccuagaugguga

SEQ ID NO: 29 - RNA, 19 nt, Artificial Sequence
  Severe acute respiratory syndrome coronavirus 2
ggaugguguuguuuguaca

SEQ ID NO: 30 - RNA, 19 nt, Artificial Sequence
  Severe acute respiratory syndrome coronavirus 2
cagcuuaugugucaaccua

SEQ ID NO: 31 - RNA, 19 nt, Artificial Sequence
  Severe acute respiratory syndrome coronavirus 2
agacaugcuuaacccuaau

SEQ ID NO: 32 - RNA, 19 nt, Artificial Sequence
  Severe acute respiratory syndrome coronavirus 2
cagagagcuagguguugua

SEQ ID NO: 33 - RNA, 19 nt, Artificial Sequence
  Severe acute respiratory syndrome coronavirus 2
guagcuggugucucuaucu

SEQ ID NO: 34 - RNA, 19 nt, Artificial Sequence
  Severe acute respiratory syndrome coronavirus 2
cugcuuaugcuaauagugu

SEQ ID NO: 35 - RNA, 19 nt, Artificial Sequence
  Severe acute respiratory syndrome coronavirus 2
ggaccucaugaauuuugcu

SEQ ID NO: 36 - RNA, 19 nt, Artificial Sequence
  Severe acute respiratory syndrome coronavirus 2
ccggcuguuuuguagauga

SEQ ID NO: 37 - RNA, 19 nt, Artificial Sequence
  Severe acute respiratory syndrome coronavirus 2
ccaccagauuugcaucugu

SEQ ID NO: 38 - RNA, 19 nt, Artificial Sequence
  Severe acute respiratory syndrome coronavirus 2
auggagugucuccuacuaa

SEQ ID NO: 39 - RNA, 19 nt, Artificial Sequence
  Severe acute respiratory syndrome coronavirus 2
gauucaacugaaugcagca

SEQ ID NO: 40 - RNA, 19 nt, Artificial Sequence
  Severe acute respiratory syndrome coronavirus 2
cuggaauagcuguugaaca

SEQ ID NO: 41 - RNA, 19 nt, Artificial Sequence
  Severe acute respiratory syndrome coronavirus 2
auagcuguugaacaagaca

SEQ ID NO: 42 - RNA, 19 nt, Artificial Sequence
  Severe acute respiratory syndrome coronavirus 2
gcagaugcuggcuucauca

SEQ ID NO: 43 - RNA, 19 nt, Artificial Sequence
  Severe acute respiratory syndrome coronavirus 2
caagauguggucaaccaaa

SEQ ID NO: 44 - RNA, 19 nt, Artificial Sequence
  Severe acute respiratory syndrome coronavirus 2
agcaccucaugguguaguc

SEQ ID NO: 45 - RNA, 19 nt, Artificial Sequence
  Severe acute respiratory syndrome coronavirus 2
ccaguugcuguaguugucu

SEQ ID NO: 46 - RNA, 19 nt, Artificial Sequence
  Severe acute respiratory syndrome coronavirus 2
guugcuguaguugucucaa

SEQ ID NO: 47 - RNA, 19 nt, Artificial Sequence
  Severe acute respiratory syndrome coronavirus 2
ggaagagacagguacguua

SEQ ID NO: 48 - RNA, 19 nt, Artificial Sequence
  Severe acute respiratory syndrome coronavirus 2
guuacacuagccauccuua

SEQ ID NO: 49 - RNA, 19 nt, Artificial Sequence
  Severe acute respiratory syndrome coronavirus 2
cgugagucuuguaaaaccu

SEQ ID NO: 50 - RNA, 19 nt, Artificial Sequence
  Severe acute respiratory syndrome coronavirus 2
ugaacaauggaaccuagua

SEQ ID NO: 51 - RNA, 19 nt, Artificial Sequence
  Severe acute respiratory syndrome coronavirus 2
uggcuugucuuguaggcuu

SEQ ID NO: 52 - RNA, 19 nt, Artificial Sequence
  Severe acute respiratory syndrome coronavirus 2
gauguggcucagcuacuuc

SEQ ID NO: 53 - RNA, 19 nt, Artificial Sequence
  Severe acute respiratory syndrome coronavirus 2
cuacaggauuggcaacuau

SEQ ID NO: 54 - RNA, 19 nt, Artificial Sequence
  Severe acute respiratory syndrome coronavirus 2
guggacccucagauucaac

SEQ ID NO: 55 - RNA, 19 nt, Artificial Sequence
  Severe acute respiratory syndrome coronavirus 2
ucaacuggcaguaaccaga

SEQ ID NO: 56 - RNA, 19 nt, Artificial Sequence
  Severe acute respiratory syndrome coronavirus 2
aaccagaauggagaacgca

SEQ ID NO: 57 - RNA, 19 nt, Artificial Sequence
  Severe acute respiratory syndrome coronavirus 2
ccagaauggagaacgcagu

SEQ ID NO: 58 - RNA, 19 nt, Artificial Sequence
  Severe acute respiratory syndrome coronavirus 2
agagcuaccagacgaauuc

SEQ ID NO: 59 - RNA, 19 nt, Artificial Sequence
  Severe acute respiratory syndrome coronavirus 2
gagccuugaauacaccaaa

SEQ ID NO: 60 - RNA, 19 nt, Artificial Sequence
  Severe acute respiratory syndrome coronavirus 2
gaaccagcuugagagcaaa

SEQ ID NO: 61 - RNA, 19 nt, Artificial Sequence
  Severe acute respiratory syndrome coronavirus 2
gcuucagcguucuucggaa

SEQ ID NO: 62 - RNA, 19 nt, Artificial Sequence
  Severe acute respiratory syndrome coronavirus 2
uagagaacagaucuacaag

SEQ ID NO: 63 - RNA, 19 nt, Artificial Sequence
  Severe acute respiratory syndrome coronavirus 2
uuuuaaaguucguuuagag

SEQ ID NO: 64 - RNA, 19 nt, Artificial Sequence
  Severe acute respiratory syndrome coronavirus 2
aucuuuugguguauucaag

SEQ ID NO: 65 - RNA, 19 nt, Artificial Sequence
  Severe acute respiratory syndrome coronavirus 2
uguuguuggccuuuaccag

SEQ ID NO: 66 - RNA, 19 nt, Artificial Sequence
  Severe acute respiratory syndrome coronavirus 2
auuucuuagugacaguuug

SEQ ID NO: 67 - RNA, 19 nt, Artificial Sequence
  Severe acute respiratory syndrome coronavirus 2
uuugaaauuuggaucuuug

SEQ ID NO: 68 - RNA, 19 nt, Artificial Sequence
  Severe acute respiratory syndrome coronavirus 2
uucuuuuuguccuuuuuag

SEQ ID NO: 69 - RNA, 19 nt, Artificial Sequence
  Severe acute respiratory syndrome coronavirus 2
aguuuacauccugauuaug

SEQ ID NO: 70 - RNA, 19 nt, Artificial Sequence
  Severe acute respiratory syndrome coronavirus 2
aguuugaaaagcaacauug

SEQ ID NO: 71 - RNA, 19 nt, Artificial Sequence
  Severe acute respiratory syndrome coronavirus 2
agaacuuccuuccuuaaag

SEQ ID NO: 72 - RNA, 19 nt, Artificial Sequence
  Severe acute respiratory syndrome coronavirus 2
aucuugauccucauaacuc

SEQ ID NO: 73 - RNA, 19 nt, Artificial Sequence
  Severe acute respiratory syndrome coronavirus 2
ucauuugaguuauaguagg

SEQ ID NO: 74 - RNA, 19 nt, Artificial Sequence
  Severe acute respiratory syndrome coronavirus 2
ucuauucuuugcacuaaug

SEQ ID NO: 75 - RNA, 19 nt, Artificial Sequence
  Severe acute respiratory syndrome coronavirus 2
aaagacaucagcauacucc

SEQ ID NO: 76 - RNA, 19 nt, Artificial Sequence
  Severe acute respiratory syndrome coronavirus 2
uaauuaccaccaaccuuag

SEQ ID NO: 77 - RNA, 19 nt, Artificial Sequence
  Severe acute respiratory syndrome coronavirus 2
aaauaucucucucaaaagg

SEQ ID NO: 78 - RNA, 19 nt, Artificial Sequence
  Severe acute respiratory syndrome coronavirus 2
aauuaaaaccaccaaaauc

SEQ ID NO: 79 - RNA, 19 nt, Artificial Sequence
  Severe acute respiratory syndrome coronavirus 2
uuaacaagcguguuuaaag

SEQ ID NO: 80 - RNA, 19 nt, Artificial Sequence
  Severe acute respiratory syndrome coronavirus 2
uuucuuuuugaauguuuac

SEQ ID NO: 81 - RNA, 19 nt, Artificial Sequence
  Severe acute respiratory syndrome coronavirus 2
agauucauuuaaauucuug

SEQ ID NO: 82 - RNA, 19 nt, Artificial Sequence
  Severe acute respiratory syndrome coronavirus 2
auauacugcucauacuuuc

SEQ ID NO: 83 - RNA, 19 nt, Artificial Sequence
  Severe acute respiratory syndrome coronavirus 2
acuucuacuaagccacaag

SEQ ID NO: 84 - RNA, 19 nt, Artificial Sequence
  Severe acute respiratory syndrome coronavirus 2
ugaugaacacauagggcug

SEQ ID NO: 85 - RNA, 19 nt, Artificial Sequence
  Severe acute respiratory syndrome coronavirus 2
aaugcacucaagaggguag

SEQ ID NO: 86 - RNA, 19 nt, Artificial Sequence
  Severe acute respiratory syndrome coronavirus 2
cuaguagguuguucuaaug

SEQ ID NO: 87 - RNA, 19 nt, Artificial Sequence
  Severe acute respiratory syndrome coronavirus 2
caagacuaugcucaggucc

SEQ ID NO: 88 - RNA, 19 nt, Artificial Sequence
  Severe acute respiratory syndrome coronavirus 2
ucauauuaggugcaagggc

SEQ ID NO: 89 - RNA, 19 nt, Artificial Sequence
  Severe acute respiratory syndrome coronavirus 2
ucaccaucuagguggaaug

SEQ ID NO: 90 - RNA, 19 nt, Artificial Sequence
  Severe acute respiratory syndrome coronavirus 2
uguacaaacaacaccaucc

SEQ ID NO: 91 - RNA, 19 nt, Artificial Sequence
  Severe acute respiratory syndrome coronavirus 2
uagguugacacauaagcug

SEQ ID NO: 92 - RNA, 19 nt, Artificial Sequence
  Severe acute respiratory syndrome coronavirus 2
auuaggguuaagcaugucu

SEQ ID NO: 93 - RNA, 19 nt, Artificial Sequence
  Severe acute respiratory syndrome coronavirus 2
uacaacaccuagcucucug

SEQ ID NO: 94 - RNA, 19 nt, Artificial Sequence
  Severe acute respiratory syndrome coronavirus 2
agauagagacaccagcuac

SEQ ID NO: 95 - RNA, 19 nt, Artificial Sequence
  Severe acute respiratory syndrome coronavirus 2
acacuauuagcauaagcag

SEQ ID NO: 96 - RNA, 19 nt, Artificial Sequence
  Severe acute respiratory syndrome coronavirus 2
agcaaaauucaugaggucc

SEQ ID NO: 97 - RNA, 19 nt, Artificial Sequence
  Severe acute respiratory syndrome coronavirus 2
ucaucuacaaaacagccgg

SEQ ID NO: 98 - RNA, 19 nt, Artificial Sequence
  Severe acute respiratory syndrome coronavirus 2
acagaugcaaaucuggugg

SEQ ID NO: 99 - RNA, 19 nt, Artificial Sequence
  Severe acute respiratory syndrome coronavirus 2
uuaguaggagacacuccau

SEQ ID NO: 100 - RNA, 19 nt, Artificial Sequence
  Severe acute respiratory syndrome coronavirus 2
ugcugcauucaguugaauc

SEQ ID NO: 101 - RNA, 19 nt, Artificial Sequence
  Severe acute respiratory syndrome coronavirus 2
uguucaacagcuauuccag

SEQ ID NO: 102 - RNA, 19 nt, Artificial Sequence
  Severe acute respiratory syndrome coronavirus 2
ugucuuguucaacagcuau

SEQ ID NO: 103 - RNA, 19 nt, Artificial Sequence
  Severe acute respiratory syndrome coronavirus 2
ugaugaagccagcaucugc

SEQ ID NO: 104 - RNA, 19 nt, Artificial Sequence
  Severe acute respiratory syndrome coronavirus 2
uuugguugaccacaucuug

SEQ ID NO: 105 - RNA, 19 nt, Artificial Sequence
  Severe acute respiratory syndrome coronavirus 2
gacuacaccaugaggugcu

SEQ ID NO: 106 - RNA, 19 nt, Artificial Sequence
  Severe acute respiratory syndrome coronavirus 2
agacaacuacagcaacugg

SEQ ID NO: 107 - RNA, 19 nt, Artificial Sequence
  Severe acute respiratory syndrome coronavirus 2
uugagacaacuacagcaac

SEQ ID NO: 108 - RNA, 19 nt, Artificial Sequence
  Severe acute respiratory syndrome coronavirus 2
uaacguaccugucucuucc

SEQ ID NO: 109 - RNA, 19 nt, Artificial Sequence
  Severe acute respiratory syndrome coronavirus 2
uaaggauggcuaguguaac

SEQ ID NO: 110 - RNA, 19 nt, Artificial Sequence
  Severe acute respiratory syndrome coronavirus 2
agguuuuacaagacucacg

SEQ ID NO: 111 - RNA, 19 nt, Artificial Sequence
  Severe acute respiratory syndrome coronavirus 2
uacuagguuccauuguuca

SEQ ID NO: 112 - RNA, 19 nt, Artificial Sequence
  Severe acute respiratory syndrome coronavirus 2
aagccuacaagacaagcca

SEQ ID NO: 113 - RNA, 19 nt, Artificial Sequence
  Severe acute respiratory syndrome coronavirus 2
gaaguagcugagccacauc

SEQ ID NO: 114 - RNA, 19 nt, Artificial Sequence
  Severe acute respiratory syndrome coronavirus 2
auaguugccaauccuguag

SEQ ID NO: 115 - RNA, 19 nt, Artificial Sequence
  Severe acute respiratory syndrome coronavirus 2
guugaaucugaggguccac

SEQ ID NO: 116 - RNA, 19 nt, Artificial Sequence
  Severe acute respiratory syndrome coronavirus 2
ucugguuacugccaguuga

SEQ ID NO: 117 - RNA, 19 nt, Artificial Sequence
  Severe acute respiratory syndrome coronavirus 2
ugcguucuccauucugguu

SEQ ID NO: 118 - RNA, 19 nt, Artificial Sequence
  Severe acute respiratory syndrome coronavirus 2
acugcguucuccauucugg

SEQ ID NO: 119 - RNA, 19 nt, Artificial Sequence
  Severe acute respiratory syndrome coronavirus 2
gaauucgucugguagcucu

SEQ ID NO: 120 - RNA, 19 nt, Artificial Sequence
  Severe acute respiratory syndrome coronavirus 2
uuugguguauucaaggcuc

SEQ ID NO: 121 - RNA, 19 nt, Artificial Sequence
  Severe acute respiratory syndrome coronavirus 2
uuugcucucaagcugguuc

SEQ ID NO: 122 - RNA, 19 nt, Artificial Sequence
  Severe acute respiratory syndrome coronavirus 2
uuccgaagaacgcugaagc